European Patent Application EP 4 733 312 A1, published April 29, 2026. Title: ANTÍGENO MULTIEPÍTOPO, COMPOSIÇÃO IMUNOGÊNICA COMPREENDENDO O REFERIDO ANTÍGENO, KIT DE DIAGNÓSTICO DO PNEUMOCOCO, E USOS DO REFERIDO ANTÍGENO. Applicant: INSTITUTO BUTANTAN. The sequence listing filed with the application follows.

SEQUENCE LISTING (24 sequences)

SEQ ID NO: 1 - protein, 20 aa, synthetic construct
  REGION 1..20: note = NanA protein epitope
TPDGKATDYRVVVDPVKPAY

SEQ ID NO: 2 - protein, 24 aa, synthetic construct
  REGION 1..24: note = NanA protein epitope
LENATVHMEFKPDAKAPAFYNLFS

SEQ ID NO: 3 - protein, 20 aa, synthetic construct
  REGION 1..20: note = NanA protein epitope
MAVYNNTATLEGRGSDGKQF

SEQ ID NO: 4 - protein, 20 aa, synthetic construct
  REGION 1..20: note = PcsB protein epitope
MSEIVSANNKMLEQQKADKK

SEQ ID NO: 5 - protein, 24 aa, synthetic construct
  REGION 1..24: note = PcsB protein epitope
DNKISNLTAQQQEAQKQVDQIQEQ

SEQ ID NO: 6 - protein, 25 aa, synthetic construct
  REGION 1..25: note = PhtD protein epitope
AGKYTTEDGYIFDPRDITSDEGDAY

SEQ ID NO: 7 - protein, 20 aa, synthetic construct
  REGION 1..20: note = PhtD protein epitope
KVGDGYVFEENGVPRYIPAK

SEQ ID NO: 8 - protein, 20 aa, synthetic construct
  REGION 1..20: note = PhtD protein epitope
GKYYVYLKDAAHADNIRTKE

SEQ ID NO: 9 - protein, 36 aa, synthetic construct
  REGION 1..36: note = Ply protein epitope
VNFKQIYYTVSVDAVKNPGDVFQDTVTVEDLKQRGI

SEQ ID NO: 10 - protein, 20 aa, synthetic construct
  REGION 1..20: note = Ply protein epitope
QVYLKLETTSKSDEVEAAFE

SEQ ID NO: 11 - protein, 27 aa, synthetic construct
  REGION 1..27: note = PncO protein epitope
GLDLLLPSILFALPHFSSLPSLLDIFI

SEQ ID NO: 12 - protein, 20 aa, synthetic construct
  REGION 1..20: note = PncO protein epitope
LIIQNYWQFSSQIGNFVWIQ

SEQ ID NO: 13 - protein, 20 aa, synthetic construct
  REGION 1..20: note = PncO protein epitope
YSGTNFAELGIYITLFFLTP

SEQ ID NO: 14 - protein, 20 aa, synthetic construct
  REGION 1..20: note = StkP protein epitope
EKVEEGRIIRTDPGAGTGRK

SEQ ID NO: 15 - protein, 22 aa, synthetic construct
  REGION 1..22: note = StkP protein epitope
VDLNKTRVKISIYKPKTTSATP

SEQ ID NO: 16 - protein, 20 aa, synthetic construct
  REGION 1..20: note = StkP protein epitope
VTTAPAGSVEGMVVEQSPRA

SEQ ID NO: 17 - protein, 20 aa, synthetic construct
  REGION 1..20: note = PspA-F1 protein epitope
AAQRKYDEDQKKTEEKAKET

SEQ ID NO: 18 - protein, 20 aa, synthetic construct
  REGION 1..20: note = PspA-F1 protein epitope
ARRSEEEYNRLPQQQLPKAE

SEQ ID NO: 19 - protein, 31 aa, synthetic construct
  REGION 1..31: note = PspA-F2 protein epitope
KKAYEEAKKKAEDAQKKYDEGQKKTEEKARK

SEQ ID NO: 20 - protein, 23 aa, synthetic construct
  REGION 1..23: note = PspA-F2 protein epitope
EVQNAYVKYQRVQRNSRLNEKER

SEQ ID NO: 21 - protein, 512 aa, synthetic construct
  REGION 1..512: note = 20 block multiepitope antigen
MVTTAPAGSVEGMVVEQSPRAKKVDLNKTRVKISIYKPKTTSATPKKEKVEEGRIIRTDPGAGTGRKGPGPGDNKISNLTAQQQEAQKQVDQIQEQKKMSEIVSANNKMLEQQKADKKGPGPGVNFKQIYYTVSVDAVKNPGDVFQDTVTVEDLKQRGIKKQVYLKLETTSKSDEVEAAFEGPGPGLENATVHMEFKPDAKAPAFYNLFSKKMAVYNNTATLEGRGSDGKQFKKTPDGKATDYRVVVDPVKPAYGPGPGGKYYVYLKDAAHADNIRTKEKKKVGDGYVFEENGVPRYIPAKKKAGKYTTEDGYIFDPRDITSDEGDAYGPGPGLIIQNYWQFSSQIGNFVWIQKKYSGTNFAELGIYITLFFLTPKKGLDLLLPSILFALPHFSSLPSLLDIFIGPGPGAAQRKYDEDQKKTEEKAKETKKARRSEEEYNRLPQQQLPKAEGPGPGKKAYEEAKKKAEDAQKKYDEGQKKTEEKARKKKEVQNAYVKYQRVQRNSRLNEKER

SEQ ID NO: 22 - protein, 518 aa, synthetic construct
  REGION 1..518: note = 20 block multiepitope antigen
MVDLNKTRVKISIYKPKTTSATPKKEVQNAYVKYQRVQRNSRLNEKERGPGPGEKVEEGRIIRTDPGAGTGRKKKAGKYTTEDGYIFDPRDITSDEGDAYGPGPGMAVYNNTATLEGRGSDGKQFKKAAQRKYDEDQKKTEEKAKETGPGPGKVGDGYVFEENGVPRYIPAKKKQVYLKLETTSKSDEVEAAFEGPGPGVNFKQIYYTVSVDAVKNPGDVFQDTVTVEDLKQRGIKKYSGTNFAELGIYITLFFLTPKKGLDLLLPSILFALPHFSSLPSLLDIFIGPGPGLIIQNYWQFSSQIGNFVWIQKKVTTAPAGSVEGMVVEQSPRAGPGPGLENATVHMEFKPDAKAPAFYNLFSKKTPDGKATDYRVVVDPVKPAYGPGPGGKYYVYLKDAAHADNIRTKEKKMSEIVSANNKMLEQQKADKKGPGPGDNKISNLTAQQQEAQKQVDQIQEQKKARRSEEEYNRLPQQQLPKAEGPGPGKKAYEEAKKKAEDAQKKYDEGQKKTEEKARK

SEQ ID NO: 23 - protein, 517 aa, synthetic construct
  REGION 1..517: note = 20 block multiepitope antigen
MAVYNNTATLEGRGSDGKQFKKEVQNAYVKYQRVQRNSRLNEKERGPGPGEKVEEGRIIRTDPGAGTGRKKKAGKYTTEDGYIFDPRDITSDEGDAYGPGPGAAQRKYDEDQKKTEEKAKETKKVDLNKTRVKISIYKPKTTSATPGPGPGKVGDGYVFEENGVPRYIPAKKKQVYLKLETTSKSDEVEAAFEGPGPGVNFKQIYYTVSVDAVKNPGDVFQDTVTVEDLKQRGIKKYSGTNFAELGIYITLFFLTPKKGLDLLLPSILFALPHFSSLPSLLDIFIGPGPGLIIQNYWQFSSQIGNFVWIQKKVTTAPAGSVEGMVVEQSPRAGPGPGLENATVHMEFKPDAKAPAFYNLFSKKTPDGKATDYRVVVDPVKPAYGPGPGGKYYVYLKDAAHADNIRTKEKKMSEIVSANNKMLEQQKADKKGPGPGDNKISNLTAQQQEAQKQVDQIQEQKKARRSEEEYNRLPQQQLPKAEGPGPGKKAYEEAKKKAEDAQKKYDEGQKKTEEKARK

SEQ ID NO: 24 - protein, 5 aa, synthetic construct
  REGION 1..5: note = Ligante
GPGPG